European Patent Application EP 4 257 154 A1, published October 11, 2023. Title: Bioactive substance conjugate, preparation method therefor and use thereof. Applicant: MediLink Therapeutics (Suzhou) Co., Ltd. The sequence listing filed with the application follows.

SEQUENCE LISTING (60 sequences)

SEQ ID NO: 1 - protein, 246 aa, Artificial Sequence
  scFv 1D1
EGQLVESGGGLVQPGGSLRLSCAASGFTISSYWMNWVRQAPGKGLEWVANIKQDGSEKYYVDSVQGRFTISRDNAKNSLYLQMNSLRAEDTAVYYCARRMYSSGWYWGAFDMWGQGTMVTVSSGGGGSGGGGSGGGGSEIVLTQSPGTLSLSPGERATLSCRASQSVSSIYLAWNQQKPGQAPRLLIYGTFKRATGIPDRFSGSGSGTDFTLTISSLEPEDFAVYYCQQYDTSSITFGQGTRLEIK

SEQ ID NO: 2 - protein, 243 aa, Artificial Sequence
  scFv 2E3
EVQLLESGGGLVQPGGSLRLSCAASGFTFSSYAMNWVRQAPGKGLEWVSGISGSGGSTYYADSVQGRFTISRDNSKNTLYLQMNSLRAEDTAVYYCAKARSGYDYFFDYWGQGTLVTVSSGGGGSGGGGSGGGGSEIVLTQSPGTLSLSPGERATLSCRASQRISSSFLAWYQQKPGQAPSLLIYGASSRATGIPDRFSGSGSGTDFTLTISSLEPEDFAVFYCQQYSNSPLTFGGGTKVEIK

SEQ ID NO: 3 - protein, 123 aa, Artificial Sequence
  1D1-01 VH
EGQLVESGGGLVQPGGSLRLSCAASGFTISSYWMNWVRQAPGKGLEWVANIKQDGSEKYYVDSVQGRFTISRDNAKNSLYLQMNSLRAEDTAVYYCARRMYSSGWYWGAFDMWGQGTMVTVSS

SEQ ID NO: 4 - protein, 7 aa, Artificial Sequence
  1D1-01 chothia HCDR1
GFTISSY

SEQ ID NO: 5 - protein, 6 aa, Artificial Sequence
  1D1-01 chothia HCDR2
KQDGSE

SEQ ID NO: 6 - protein, 14 aa, Artificial Sequence
  1D1-01 chothia HCDR3
RMYSSGWYWGAFDM

SEQ ID NO: 7 - protein, 5 aa, Artificial Sequence
  1D1-01 kabat HCDR1
SYWMN

SEQ ID NO: 8 - protein, 17 aa, Artificial Sequence
  1D1-01 kabat HCDR2
NIKQDGSEKYYVDSVQG

SEQ ID NO: 9 - protein, 14 aa, Artificial Sequence
  1D1-01 kabat HCDR3
RMYSSGWYWGAFDM

SEQ ID NO: 10 - protein, 8 aa, Artificial Sequence
  1D1-01 IMGT HCDR1
GFTISSYW

SEQ ID NO: 11 - protein, 8 aa, Artificial Sequence
  1D1-01 IMGT HCDR2
IKQDGSEK

SEQ ID NO: 12 - protein, 16 aa, Artificial Sequence
  1D1-01 IMGT HCDR3
ARRMYSSGWYWGAFDM

SEQ ID NO: 13 - protein, 108 aa, Artificial Sequence
  1D1-01 VL
EIVLTQSPGTLSLSPGERATLSCRASQSVSSIYLAWNQQKPGQAPRLLIYGTFKRATGIPDRFSGSGSGTDFTLTISSLEPEDFAVYYCQQYDTSSITFGQGTRLEIK

SEQ ID NO: 14 - protein, 12 aa, Artificial Sequence
  1D1-01 chothia LCDR1
RASQSVSSIYLA

SEQ ID NO: 15 - protein, 7 aa, Artificial Sequence
  1D1-01 chothia LCDR2
GTFKRAT

SEQ ID NO: 16 - protein, 9 aa, Artificial Sequence
  1D1-01 chothia LCDR3
QQYDTSSIT

SEQ ID NO: 17 - protein, 12 aa, Artificial Sequence
  1D1-01 kabat LCDR1
RASQSVSSIYLA

SEQ ID NO: 18 - protein, 7 aa, Artificial Sequence
  1D1-01 kabat LCDR2
GTFKRAT

SEQ ID NO: 19 - protein, 9 aa, Artificial Sequence
  1D1-01 kabat LCDR3
QQYDTSSIT

SEQ ID NO: 20 - protein, 7 aa, Artificial Sequence
  1D1-01 IMGT LCDR1
QSVSSIY

SEQ ID NO: 21 - protein, 9 aa, Artificial Sequence
  202-2-1 Kabat/IMGT LCDR3
QQLNSYPLT

SEQ ID NO: 22 - protein, 9 aa, Artificial Sequence
  1D1-01 IMGT LCDR3
QQYDTSSIT

SEQ ID NO: 23 - protein, 120 aa, Artificial Sequence
  2E3-02 VH
EVQLLESGGGLVQPGGSLRLSCAASGFTFSSYAMNWVRQAPGKGLEWVSGISGSGGSTYYADSVQGRFTISRDNSKNTLYLQMNSLRAEDTAVYYCAKARSGYDYFFDYWGQGTLVTVSS

SEQ ID NO: 24 - protein, 7 aa, Artificial Sequence
  2E3-02 chothia HCDR1
GFTFSSY

SEQ ID NO: 25 - protein, 6 aa, Artificial Sequence
  2E3-02 chothia HCDR2
SGSGGS

SEQ ID NO: 26 - protein, 11 aa, Artificial Sequence
  2E3-02 chothia HCDR3
ARSGYDYFFDY

SEQ ID NO: 27 - protein, 5 aa, Artificial Sequence
  2E3-02 kabat HCDR1
SYAMN

SEQ ID NO: 28 - protein, 17 aa, Artificial Sequence
  2E3-02 kabat HCDR2
GISGSGGSTYYADSVQG

SEQ ID NO: 29 - protein, 11 aa, Artificial Sequence
  2E3-02 kabat HCDR3
ARSGYDYFFDY

SEQ ID NO: 30 - protein, 8 aa, Artificial Sequence
  2E3-02 IMGT HCDR1
GFTFSSYA

SEQ ID NO: 31 - protein, 8 aa, Artificial Sequence
  2E3-02 IMGT HCDR2
ISGSGGST

SEQ ID NO: 32 - protein, 13 aa, Artificial Sequence
  2E3-02 IMGT HCDR3
AKARSGYDYFFDY

SEQ ID NO: 33 - protein, 108 aa, Artificial Sequence
  2E3-02 VL
EIVLTQSPGTLSLSPGERATLSCRASQRISSSFLAWYQQKPGQAPSLLIYGASSRATGIPDRFSGSGSGTDFTLTISSLEPEDFAVFYCQQYSNSPLTFGGGTKVEIK

SEQ ID NO: 34 - protein, 12 aa, Artificial Sequence
  2E3-02 chothia LCDR1
RASQRISSSFLA

SEQ ID NO: 35 - protein, 7 aa, Artificial Sequence
  2E3-02 chothia LCDR2
GASSRAT

SEQ ID NO: 36 - protein, 9 aa, Artificial Sequence
  2E3-02 chothia LCDR3
QQYSNSPLT

SEQ ID NO: 37 - protein, 12 aa, Artificial Sequence
  2E3-02 kabat LCDR1
RASQRISSSFLA

SEQ ID NO: 38 - protein, 7 aa, Artificial Sequence
  2E3-02 kabat LCDR2
GASSRAT

SEQ ID NO: 39 - protein, 9 aa, Artificial Sequence
  2E3-02 kabat LCDR3
QQYSNSPLT

SEQ ID NO: 40 - protein, 7 aa, Artificial Sequence
  2E3-02  IMGT LCDR1
QRISSSF

SEQ ID NO: 41 - protein, 6 aa, Artificial Sequence
  202-2-1 IMGT LCDR1
QGISSY

SEQ ID NO: 42 - protein, 9 aa, Artificial Sequence
  2E3-02 IMGT LCDR3
QQYSNSPLT

SEQ ID NO: 43 - protein, 330 aa, Artificial Sequence [sequence omitted]

SEQ ID NO: 44 - protein, 107 aa, Artificial Sequence [sequence omitted]

SEQ ID NO: 45 - protein, 453 aa, Artificial Sequence
  1D1-01 HC
EGQLVESGGGLVQPGGSLRLSCAASGFTISSYWMNWVRQAPGKGLEWVANIKQDGSEKYYVDSVQGRFTISRDNAKNSLYLQMNSLRAEDTAVYYCARRMYSSGWYWGAFDMWGQGTMVTVSSASTKGPSVFPLAPSSKSTSGGTAALGCLVKDYFPEPVTVSWNSGALTSGVHTFPAVLQSSGLYSLSSVVTVPSSSLGTQTYICNVNHKPSNTKVDKKVEPKSCDKTHTCPPCPAPELLGGPSVFLFPPKPKDTLMISRTPEVTCVVVDVSHEDPEVKFNWYVDGVEVHNAKTKPREEQYNSTYRVVSVLTVLHQDWLNGKEYKCKVSNKALPAPIEKTISKAKGQPREPQVYTLPPSRDELTKNQVSLTCLVKGFYPSDIAVEWESNGQPENNYKTTPPVLDSDGSFFLYSKLTVDKSRWQQGNVFSCSVMHEALHNHYTQKSLSLSPGK

SEQ ID NO: 46 - protein, 215 aa, Artificial Sequence
  1D1-01 LC
EIVLTQSPGTLSLSPGERATLSCRASQSVSSIYLAWNQQKPGQAPRLLIYGTFKRATGIPDRFSGSGSGTDFTLTISSLEPEDFAVYYCQQYDTSSITFGQGTRLEIKRTVAAPSVFIFPPSDEQLKSGTASVVCLLNNFYPREAKVQWKVDNALQSGNSQESVTEQDSKDSTYSLSSTLTLSKADYEKHKVYACEVTHQGLSSPVTKSFNRGEC

SEQ ID NO: 47 - protein, 450 aa, Artificial Sequence
  2E3-02 HC
EVQLLESGGGLVQPGGSLRLSCAASGFTFSSYAMNWVRQAPGKGLEWVSGISGSGGSTYYADSVQGRFTISRDNSKNTLYLQMNSLRAEDTAVYYCAKARSGYDYFFDYWGQGTLVTVSSASTKGPSVFPLAPSSKSTSGGTAALGCLVKDYFPEPVTVSWNSGALTSGVHTFPAVLQSSGLYSLSSVVTVPSSSLGTQTYICNVNHKPSNTKVDKKVEPKSCDKTHTCPPCPAPELLGGPSVFLFPPKPKDTLMISRTPEVTCVVVDVSHEDPEVKFNWYVDGVEVHNAKTKPREEQYNSTYRVVSVLTVLHQDWLNGKEYKCKVSNKALPAPIEKTISKAKGQPREPQVYTLPPSRDELTKNQVSLTCLVKGFYPSDIAVEWESNGQPENNYKTTPPVLDSDGSFFLYSKLTVDKSRWQQGNVFSCSVMHEALHNHYTQKSLSLSPGK

SEQ ID NO: 48 - protein, 215 aa, Artificial Sequence
  2E3-02 LC
EIVLTQSPGTLSLSPGERATLSCRASQRISSSFLAWYQQKPGQAPSLLIYGASSRATGIPDRFSGSGSGTDFTLTISSLEPEDFAVFYCQQYSNSPLTFGGGTKVEIKRTVAAPSVFIFPPSDEQLKSGTASVVCLLNNFYPREAKVQWKVDNALQSGNSQESVTEQDSKDSTYSLSSTLTLSKADYEKHKVYACEVTHQGLSSPVTKSFNRGEC

SEQ ID NO: 49 - protein, 119 aa, Artificial Sequence
  202-2-1 VH
EVQLVESGGGVVQPGRSLRLSCAASGFTFSTYGMHWVRQAPGKGLEWVAVIWYDVSHKYYADSVKGRFTISRDNSKNTLSLQMNSLRAEDTAVYYCARDWGDPDAFDIWGQGTMVTVSS

SEQ ID NO: 50 - protein, 107 aa, Artificial Sequence
  202-2-1 VL
DIQLTQSPSFLSASVGDRVTITCRASQGISSYLAWYQQKPGKAPKLLIYAASTLQSGVPSRFSGSGSGTEFTLTISSLQPEDFATYYCQQLNSYPLTFGGGTKVEIK

SEQ ID NO: 51 - protein, 449 aa, Artificial Sequence
  202-2-1 HC
EVQLVESGGGVVQPGRSLRLSCAASGFTFSTYGMHWVRQAPGKGLEWVAVIWYDVSHKYYADSVKGRFTISRDNSKNTLSLQMNSLRAEDTAVYYCARDWGDPDAFDIWGQGTMVTVSSASTKGPSVFPLAPSSKSTSGGTAALGCLVKDYFPEPVTVSWNSGALTSGVHTFPAVLQSSGLYSLSSVVTVPSSSLGTQTYICNVNHKPSNTKVDKKVEPKSCDKTHTCPPCPAPELLGGPSVFLFPPKPKDTLMISRTPEVTCVVVDVSHEDPEVKFNWYVDGVEVHNAKTKPREEQYNSTYRVVSVLTVLHQDWLNGKEYKCKVSNKALPAPIEKTISKAKGQPREPQVYTLPPSRDELTKNQVSLTCLVKGFYPSDIAVEWESNGQPENNYKTTPPVLDSDGSFFLYSKLTVDKSRWQQGNVFSCSVMHEALHNHYTQKSLSLSPGK

SEQ ID NO: 52 - protein, 214 aa, Artificial Sequence
  202-2-1 LC
DIQLTQSPSFLSASVGDRVTITCRASQGISSYLAWYQQKPGKAPKLLIYAASTLQSGVPSRFSGSGSGTEFTLTISSLQPEDFATYYCQQLNSYPLTFGGGTKVEIKRTVAAPSVFIFPPSDEQLKSGTASVVCLLNNFYPREAKVQWKVDNALQSGNSQESVTEQDSKDSTYSLSSTLTLSKADYEKHKVYACEVTHQGLSSPVTKSFNRGEC

SEQ ID NO: 53 - protein, 5 aa, Artificial Sequence
  202-2-1 Kabat HCDR1
TYGMH

SEQ ID NO: 54 - protein, 17 aa, Artificial Sequence
  202-2-1 Kabat HCDR2
VIWYDVSHKYYADSVKG

SEQ ID NO: 55 - protein, 10 aa, Artificial Sequence
  202-2-1 Kabat HCDR3
DWGDPDAFDI

SEQ ID NO: 56 - protein, 8 aa, Artificial Sequence
  202-2-1 IMGT HCDR1
GFTFSTYG

SEQ ID NO: 57 - protein, 8 aa, Artificial Sequence
  202-2-1 IMGT HCDR2
IWYDVSHK

SEQ ID NO: 58 - protein, 12 aa, Artificial Sequence
  202-2-1 IMGT HCDR3
ARDWGDPDAFDI

SEQ ID NO: 59 - protein, 11 aa, Artificial Sequence
  202-2-1 Kabat LCDR1
RASQGISSYLA

SEQ ID NO: 60 - protein, 7 aa, Artificial Sequence
  202-2-1 Kabat LCDR2
AASTLQS